European Patent Specification EP 3 715 449 B1, published March 13, 2024. Title: Novel lactic acid bacteria and use thereof. Applicant: UNIVERSITY-INDUSTRY COOPERATION GROUP OF KYUNG HEE UNIVERSITY. The sequence listing filed with the application follows.

SEQUENCE LISTING (2 sequences)

SEQ ID NO: 1 - DNA, 1513 bp, Artificial Sequence
  NK41 16s rDNA
agattcaccctaatcatctgccccaccttaggcggctagctccccgaagggttaccccaccgactttgggtgttgcaaactctcatggtgtgacgggcggtgtgtacaaggccccgggaacgtatttccacccgggcatgctgatccgcgattactagcgattccgacttcgtgcaggcgagttgcagcctgcagtccgaactgagaacggttttaagagattagcttgccctcgcgagttcgcgactcgttgtaccgtccattgtagcacgtgtgtagcccaggtcataaggggcatgatgatctgacgtcgtccccaccttcctccggtttgtcaccggcagtctcactagagtgcccaactgaatgctggcaactagtaacaagggttgcgctcgttgcgggacttaacccaacatctcacgacacgagctgacgacgaccatgcaccacctgtcattgcgttcccgaaggaaacgccctatctctagggttggcgcaagatgtcaagacctggtaaggttcttcgcgtagcttcgaattaaaccacatgctccaccgcttgtgcgggcccccgtcaattcctttgagtttcaaccttgcggtcgtactccccaggcggagtgcttaatgcgttagctgcggcactgaagggcggaaaccctccaacacctagcactcatcgtttacggcatggactaccagggtatctaatcctgttcgctacccatgctttcgagcctcagcgtcagttgcagaccagacagccgccttcgccactggtgttcttccatatatctacgcattccaccgctacacatggagttccactgtcctcttctgcactcaagtctgacagtttccgatgcacttctttggttaagccaaaggctttcacatcagacttatcaaaccgcctgcgctcgctttacgcccaataaatccggataacgcttgccacctacgtattaccgcggctgctggcacgtagttagccgtgactttctggttagataccgtcactgcgtgaacagttgctctcacgcacgttcttctctaacaacagagctttacgagccgaaacccttcttcactcacgcggtgttgctccatcaggcttgcgcccattgtggaagattccctactgctgcctcccgtaggagtatggaccgtgtctcagttccattgtggccgatcagtctctcaactcggctacgcatcacagccttggtaggccgttaccctaccaacaagctaatgcgccgcaggtccatcccaaagtgatagccgaagccatcttttaaatttgaatcatgcgattcaaattgttatgcggtattagcatctgtttccaaatgttatcccccgctttggggcaggttacctacgtgttactcacccgtccgccactcgctggtaaaccaacgtcaagtccgtgcaagcacgttcaatcagttgggccaacgcgttcgacttgcatgtattaggcacaccgccggcgttcatcctgagc

SEQ ID NO: 2 - DNA, 1469 bp, Artificial Sequence
  NK46 16s rDNA
tttacccctgttacgacttagtcccaatcacgagcctcaccttagacggctccatcccacaaggggttaggccaccggcttcgggtgctgcccactttcatgacttgacgggcggtgtgtacaaggcccgggaacgcattcaccgcgacgttgctgattcgcgattactagcgactccgccttcacgcagtcgagttgcagactgcgatccgaactgagaccggttttcagggatccgctccgcgtcgccgcgtcgcatcccgttgtaccggccattgtagcatgcgtgaagccctggacgtaaggggcatgatgatctgacgtcatccccaccttcctccgagttaaccccggcggtcccccgtgagttcccggcataatccgctggcaacacggggcgagggttgcgctcgttgcgggacttaacccaacatctcacgacacgagctgacgacgaccatgcaccacctgtgaacccgccccgaagggaagccgcatctctacgaccgtcgggaacatgtcaagcccaggtaaggttcttcgcgttgcatcgaattaatccgcatgctccgccgcttgtgcgggcccccgtcaatttctttgagttttagccttgcggccgtactccccaggcgggatgcttaacgcgttagctccgacacggaacccgtggaacgggccccacatccagcatccaccgtttacggcgtggactaccagggtatctaatcctgttcgctccccacgctttcgctcctcagcgtcagtaacggcccagagacctgccttcgccattggtgttcttcccgatatctacacattccaccgttacaccgggaattccagtctcccctaccgcactcaagcccgcccgtacccggcgcggatccaccgttaagcgatggactttcacaccggacgcgacgaaccgcctacgagccctttacgcccaataattccggataacgcttgcaccctacgtattaccgcggctgctggcacgtagttagccggtgcttattcaacgggtaaactcactctcgcttgctccccgataaaagaggtttacaacccgaaggcctccatccctcacgcggcgtcgctgcatcaggcttgcgcccattgtgcaatattccccactgctgcctcccgtaggagtctgggccgtatctcagtcccaatgtggccggtcgccctctcaggccggctacccgtcgaagccacggtgggccgttaccccgccgtcaagctgataggacgcgaccccatcccataccgcgaaagctttcccagaagaccatgcgatcaactggagcatccggcattaccacccgtttccaggagctattccggtgtatggggcaggtcggtcacgcattactcacccgttcgccactctcaccaccaagcaaagcctgatggatcccgttcgacttgcatgtgttaagcacgccgccagcgttcatcct